European Patent Specification EP 3 123 090 B1, published September 23, 2026. Title: LYOPHILIZED FACTOR IX FORMULATIONS. Applicant: BIOGEN IDEC MA INC. Thome, Brian M. Parkhurst-Lang, Cherie Leveille, Brandon W. Application To be filed. The sequence listing filed with the application follows.

SEQUENCE LISTING (14 sequences)

SEQ ID NO: 1 - DNA, 7583 bp, Artificial Sequence
  FIX-Fc Chain
gcgcgcgttgacattgattattgactagttattaatagtaatcaattacggggtcattagttcatagcccatatatggagttccgcgttacataacttacggtaaatggcccgcctggctgaccgcccaacgacccccgcccattgacgtcaataatgacgtatgttcccatagtaacgccaatagggactttccattgacgtcaatgggtggagtatttacggtaaactgcccacttggcagtacatcaagtgtatcatatgccaagtacgccccctattgacgtcaatgacggtaaatggcccgcctggcattatgcccagtacatgaccttatgggactttcctacttggcagtacatctacgtattagtcatcgctattaccatggtgatgcggttttggcagtacatcaatgggcgtggatagcggtttgactcacggggatttccaagtctccaccccattgacgtcaatgggagtttgttttggcaccaaaatcaacgggactttccaaaatgtcgtaacaactccgccccattgacgcaaatgggcggtaggcgtgtacggtgggaggtctatataagcagagctctctggctaactagagaacccactgcttactggcttatcgaaattaatacgactcactatagggagacccaagcttcgcgacgtacggccgccaccatgcagcgcgtgaacatgatcatggcagaatcaccaggcctcatcaccatctgccttttaggatatctactcagtgctgaatgtacaggtttgtttccttttttaaaatacattgagtatgcttgccttttagatatagaaatatctgatgctgtcttcttcactaaattttgattacatgatttgacagcaatattgaagagtctaacagccagcacgcaggttggtaagtactgtgggaacatcacagattttggctccatgccctaaagagaaattggctttcagattatttggattaaaaacaaagactttcttaagagatgtaaaattttcatgatgttttcttttttgctaaaactaaagaattattcttttacatttcagtttttcttgatcatgaaaacgccaacaaaattctgaatcggccaaagaggtataattcaggtaaattggaagagtttgttcaagggaatctagagagagaatgtatggaagaaaagtgtagttttgaagaagcacgagaagtttttgaaaacactgaaagaacaactgaattttggaagcagtatgttgatggagatcagtgtgagtccaatccatgtttaaatggcggcagttgcaaggatgacattaattcctatgaatgttggtgtccctttggatttgaaggaaagaactgtgaattagatgtaacatgtaacattaagaatggcagatgcgagcagttttgtaaaaatagtgctgataacaaggtggtttgctcctgtactgagggatatcgacttgcagaaaaccagaagtcctgtgaaccagcagtgccatttccatgtggaagagtttctgtttcacaaacttctaagctcacccgtgctgagactgtttttcctgatgtggactatgtaaattctactgaagctgaaaccattttggataacatcactcaaagcacccaatcatttaatgacttcactcgggttgttggtggagaagatgccaaaccaggtcaattcccttggcaggttgttttgaatggtaaagttgatgcattctgtggaggctctatcgttaatgaaaaatggattgtaactgctgcccactgtgttgaaactggtgttaaaattacagttgtcgcaggtgaacataatattgaggagacagaacatacagagcaaaagcgaaatgtgattcgaattattcctcaccacaactacaatgcagctattaataagtacaaccatgacattgcccttctggaactggacgaacccttagtgctaaacagctacgttacacctatttgcattgctgacaaggaatacacgaacatcttcctcaaatttggatctggctatgtaagtggctggggaagagtcttccacaaagggagatcagctttagttcttcagtaccttagagttccacttgttgaccgagccacatgtcttcgatctacaaagttcaccatctataacaacatgttctgtgctggcttccatgaaggaggtagagattcatgtcaaggagatagtgggggaccccatgttactgaagtggaagggaccagtttcttaactggaattattagctggggtgaagagtgtgcaatgaaaggcaaatatggaatatataccaaggtgtcccggtatgtcaactggattaaggaaaaaacaaagctcactgacaaaactcacacatgcccaccgtgcccagctccggaactcctgggcggaccgtcagtcttcctcttccccccaaaacccaaggacaccctcatgatctcccggacccctgaggtcacatgcgtggtggtggacgtgagccacgaagaccctgaggtcaagttcaactggtacgtggacggcgtggaggtgcataatgccaagacaaagccgcgggaggagcagtacaacagcacgtaccgtgtggtcagcgtcctcaccgtcctgcaccaggactggctgaatggcaaggagtacaagtgcaaggtctccaacaaagccctcccagcccccatcgagaaaaccatctccaaagccaaagggcagccccgagaaccacaggtgtacaccctgcccccatcccgggatgagctgaccaagaaccaggtcagcctgacctgcctggtcaaaggcttctatcccagcgacatcgccgtggagtgggagagcaatgggcagccggagaacaactacaagaccacgcctcccgtgttggactccgacggctccttcttcctctacagcaagctcaccgtggacaagagcaggtggcagcaggggaacgtcttctcatgctccgtgatgcatgaggctctgcacaaccactacacgcagaagagcctctccctgtctccgggtaaatgagaattcagacatgataagatacattgatgagtttggacaaaccacaactagaatgcagtgaaaaaaatgctttatttgtgaaatttgtgatgctattgctttatttgtaaccattataagctgcaataaacaagttggggtgggcgaagaactccagcatgagatccccgcgctggaggatcatccagccggcgtcccggaaaacgattccgaagcccaacctttcatagaaggcggcggtggaatcgaaatctcgtagcacgtgtcagtcctgctcctcggccacgaagtgcacgcagttgccggccgggtcgcgcagggcgaactcccgcccccacggctgctcgccgatctcggtcatggccggcccggaggcgtcccggaagttcgtggacacgacctccgaccactcggcgtacagctcgtccaggccgcgcacccacacccaggccagggtgttgtccggcaccacctggtcctggaccgcgctgatgaacagggtcacgtcgtcccggaccacaccggcgaagtcgtcctccacgaagtcccgggagaacccgagccggtcggtccagaactcgaccgctccggcgacgtcgcgcgcggtgagcaccggaacggcactggtcaacttggccatggtttagttcctcaccttgtcgtattatactatgccgatatactatgccgatgattaattgtcaacacgtgctgatcagatccgaaaatggatatacaagctcccgggagctttttgcaaaagcctaggcctccaaaaaagcctcctcactacttctggaatagctcagaggcagaggcggcctcggcctctgcataaataaaaaaaattagtcagccatggggcggagaatgggcggaactgggcggagttaggggcgggatgggcggagttaggggcgggactatggttgctgactaattgagatgcatgctttgcatacttctgcctgctggggagcctggggactttccacacctggttgctgactaattgagatgcatgctttgcatacttctgcctgctggggagcctggggactttccacaccctcgtcgagctagcttcgtgaggctccggtgcccgtcagtgggcagagcgcacatcgcccacagtccccgagaagttggggggaggggtcggcaattgaaccggtgcctagagaaggtggcgcggggtaaactgggaaagtgatgtcgtgtactggctccgcctttttcccgagggtgggggagaaccgtatataagtgcagtagtcgccgtgaacgttctttttcgcaacgggtttgccgccagaacacaggtaagtgccgtgtgtggttcccgcgggcctggcctctttacgggttatggcccttgcgtgccttgaattacttccacctggctccagtacgtgattcttgatcccgagctggagccaggggcgggccttgcgctttaggagccccttcgcctcgtgcttgagttgaggcctggcctgggcgctggggccgccgcgtgcgaatctggtggcaccttcgcgcctgtctcgctgctttcgataagtctctagccatttaaaatttttgatgacctgctgcgacgctttttttctggcaagatagtcttgtaaatgcgggccaggatctgcacactggtatttcggtttttggggccgcgggcggcgacggggcccgtgcgtcccagcgcacatgttcggcgaggcggggcctgcgagcgcggccaccgagaatcggacgggggtagtctcaagctggccggcctgctctggtgcctggcctcgcgccgccgtgtatcgccccgccctgggcggcaaggctggcccggtcggcaccagttgcgtgagcggaaagatggccgcttcccggccctgctccagggggctcaaaatggaggacgcggcgctcgggagagcgggcgggtgagtcacccacacaaaggaaaggggcctttccgtcctcagccgtcgcttcatgtgactccacggagtaccgggcgccgtccaggcacctcgattagttctggagcttttggagtacgtcgtctttaggttggggggaggggttttatgcgatggagtttccccacactgagtgggtggagactgaagttaggccagcttggcacttgatgtaattctccttggaatttgccctttttgagtttggatcttggttcattctcaagcctcagacagtggttcaaagtttttttcttccatttcaggtgtcgtgaacacgtggtcgcggccgcgccgccaccatggagacagacacactcctgctatgggtactgctgctctgggttccaggttccactggtgacaaaactcacacatgcccaccgtgcccagcacctgaactcctgggaggaccgtcagtcttcctcttccccccaaaacccaaggacaccctcatgatctcccggacccctgaggtcacatgcgtggtggtggacgtgagccacgaagaccctgaggtcaagttcaactggtacgtggacggcgtggaggtgcataatgccaagacaaagccgcgggaggagcagtacaacagcacgtaccgtgtggtcagcgtcctcaccgtcctgcaccaggactggctgaatggcaaggagtacaagtgcaaggtctccaacaaagccctcccagcccccatcgagaaaaccatctccaaagccaaagggcagccccgagaaccacaggtgtacaccctgcccccatcccgcgatgagctgaccaagaaccaggtcagcctgacctgcctggtcaaaggcttctatcccagcgacatcgccgtggagtgggagagcaatgggcagccggagaacaactacaagaccacgcctcccgtgttggactccgacggctccttcttcctctacagcaagctcaccgtggacaagagcaggtggcagcaggggaacgtcttctcatgctccgtgatgcatgaggctctgcacaaccactacacgcagaagagcctctccctgtctccgggtaaatgactcgagagatctggccggctgggcccgtttcgaaggtaagcctatccctaaccctctcctcggtctcgattctacgcgtaccggtcatcatcaccatcaccattgagtttaaacccgctgatcagcctcgactgtgccttctagttgccagccatctgttgtttgcccctcccccgtgccttccttgaccctggaaggtgccactcccactgtcctttcctaataaaatgaggaaattgcatcgcattgtctgagtaggtgtcattctattctggggggtggggtggggcaggacagcaagggggaggattgggaagacaatagcaggcatgctggggatgcggtgggctctatggcttctgaggcggaaagaaccagtggcggtaatacggttatccacagaatcaggggataacgcaggaaagaacatgtgagcaaaaggccagcaaaaggccaggaaccgtaaaaaggccgcgttgctggcgtttttccataggctccgcccccctgacgagcatcacaaaaatcgacgctcaagtcagaggtggcgaaacccgacaggactataaagataccaggcgtttccccctagaagctccctcgtgcgctctcctgttccgaccctgccgcttaccggatacctgtccgcctttctcccttcgggaagcgtggcgctttctcatagctcacgctgtaggtatctcagttcggtgtaggtcgttcgctccaagctgggctgtgtgcacgaaccccccgttcagcccgaccgctgcgccttatccggtaactatcgtcttgagtccaacccggtaagacacgacttatcgccactggcagcagccactggtaacaggattagcagagcgaggtatgtaggcggtgctacagagttcttgaagtggtggcctaactacggctacactagaagaacagtatttggtatctgcgctctgctgaagccagttaccttcggaaaaagagttggtagctcttgatccggcaaacaaaccaccgctggtagcggtggtttttttgtttgcaagcagcagattacgcgcagaaaaaaaggatctcaagaagatcctttgatcttttctacggggtctgacgctcagtggaacgaaaactcacgttaagggattttggtcatgacattaacctataaaaataggcgtatcacgaggccctttcgtctcgcgcgtttcggtgatgacggtgaaaacctctgacacatgcagctcccggagacggtcacagcttgtctgtaagcggatgccgggagcagacaagcccgtcagggcgcgtcagcgggtgttggcgggtgtcggggctggcttaactatgcggcatcagagcagattgtactgagagtgcaccatatatgcggtgtgaaataccgcacagatgcgtaaggagaaaataccgcatcaggcgccattcgccattcaggctgcgcaactgttgggaagggcgatcggtgcgggcctcttcgctattacgcca

SEQ ID NO: 2 - protein, 642 aa, Artificial Sequence
  FIX-Fc Chain
YNSGKLEEFVQGNLERECMEEKCSFEEAREVFENTERTTEFWKQYVDGDQCESNPCLNGGSCKDDINSYECWCPFGFEGKNCELDVTCNIKNGRCEQFCKNSADNKVVCSCTEGYRLAENQKSCEPAVPFPCGRVSVSQTSKLTRAETVFPDVDYVNSTEAETILDNITQSTQSFNDFTRVVGGEDAKPGQFPWQVVLNGKVDAFCGGSIVNEKWIVTAAHCVETGVKITVVAGEHNIEETEHTEQKRNVIRIIPHHNYNAAINKYNHDIALLELDEPLVLNSYVTPICIADKEYTNIFLKFGSGYVSGWGRVFHKGRSALVLQYLRVPLVDRATCLRSTKFTIYNNMFCAGFHEGGRDSCQGDSGGPHVTEVEGTSFLTGIISWGEECAMKGKYGIYTKVSRYVNWIKEKTKLTDKTHTCPPCPAPELLGGPSVFLFPPKPKDTLMISRTPEVTCVVVDVSHEDPEVKFNWYVDGVEVHNAKTKPREEQYNSTYRVVSVLTVLHQDWLNGKEYKCKVSNKALPAPIEKTISKAKGQPREPQVYTLPPSRDELTKNQVSLTCLVKGFYPSDIAVEWESNGQPENNYKTTPPVLDSDGSFFLYSKLTVDKSRWQQGNVFSCSVMHEALHNHYTQKSLSLSPGK

SEQ ID NO: 3 - DNA, 741 bp, Artificial Sequence
  Fc Portion
atggagacagacacactcctgctatgggtactgctgctctgggttccaggttccactggtgacaaaactcacacatgcccaccgtgcccagcacctgaactcctgggaggaccgtcagtcttcctcttccccccaaaacccaaggacaccctcatgatctcccggacccctgaggtcacatgcgtggtggtggacgtgagccacgaagaccctgaggtcaagttcaactggtacgtggacggcgtggaggtgcataatgccaagacaaagccgcgggaggagcagtacaacagcacgtaccgtgtggtcagcgtcctcaccgtcctgcaccaggactggctgaatggcaaggagtacaagtgcaaggtctccaacaaagccctcccagcccccatcgagaaaaccatctccaaagccaaagggcagccccgagaaccacaggtgtacaccctgcccccatcccgcgatgagctgaccaagaaccaggtcagcctgacctgcctggtcaaaggcttctatcccagcgacatcgccgtggagtgggagagcaatgggcagccggagaacaactacaagaccacgcctcccgtgttggactccgacggctccttcttcctctacagcaagctcaccgtggacaagagcaggtggcagcaggggaacgtcttctcatgctccgtgatgcatgaggctctgcacaaccactacacgcagaagagcctctccctgtctccgggtaaa

SEQ ID NO: 4 - protein, 227 aa, Artificial Sequence
  Fc Portion
DKTHTCPPCPAPELLGGPSVFLFPPKPKDTLMISRTPEVTCVVVDVSHEDPEVKFNWYVDGVEVHNAKTKPREEQYNSTYRVVSVLTVLHQDWLNGKEYKCKVSNKALPAPIEKTISKAKGQPREPQVYTLPPSRDELTKNQVSLTCLVKGFYPSDIAVEWESNGQPENNYKTTPPVLDSDGSFFLYSKLTVDKSRWQQGNVFSCSVMHEALHNHYTQKSLSLSPGK

SEQ ID NO: 5 - protein, 11 aa, Artificial Sequence
  Core sequence of albumin-binding peptides
DICLPRWGCLW

SEQ ID NO: 6 - protein, 32 aa, Artificial Sequence
  CTP peptide
DPRFQDSSSSKAPPPSLPSPSRLPGPSDTPIL

SEQ ID NO: 7 - protein, 28 aa, Artificial Sequence
  CTP peptide
SSSSKAPPPSLPSPSRLPGPSDTPILPQ

SEQ ID NO: 8 - protein, 20 aa, Artificial Sequence
  PAS peptide
ASPAAPAPASPAAPAPSAPA

SEQ ID NO: 9 - protein, 20 aa, Artificial Sequence
  PAS peptide
AAPASPAPAAPSAPAPAAPS

SEQ ID NO: 10 - protein, 20 aa, Artificial Sequence
  PAS peptide
APSSPSPSAPSSPSPASPSS

SEQ ID NO: 11 - protein, 19 aa, Artificial Sequence
  PAS peptide
APSSPSPSAPSSPSPASPS

SEQ ID NO: 12 - protein, 20 aa, Artificial Sequence
  PAS peptide
SSPSAPSPSSPASPSPSSPA

SEQ ID NO: 13 - protein, 24 aa, Artificial Sequence
  PAS peptide
AASPAAPSAPPAAASPAAPSAPPA

SEQ ID NO: 14 - protein, 20 aa, Artificial Sequence
  PAS peptide
ASAAAPAAASAAASAPSAAA